European Patent Specification EP 3 535 242 B1, published January 24, 2024. Title: DNA PRIMASE AND GYRASE INHIBITORS. Applicant: B. G. NEGEV TECHNOLOGIES AND APPLICATIONS LTD., AT BEN-GURION UNIVERSITY. The sequence listing filed with the application follows.

SEQUENCE LISTING (4 sequences)

SEQ ID NO: 1 - protein, 82 aa, Aquifex aeolicus
GFAILVEGYFDLLRLFSALTQNQANLLSKFTKKVYILYDGDDAGRKAMKSAIPLLLSAGVEVYPVYLPEGEGIRNVVAPLGT

SEQ ID NO: 2 - protein, 82 aa, Staphylococcus aureus
DEIVLLEGFMDVIKSDTAGLKNVVATMGTQLSDEHITFIRKLTSNITLMFDGDFAGSEATLKTGQHLLQQGLNVFVIQLPSG

SEQ ID NO: 3 - protein, 89 aa, Bacteriophage T7
KKIVVTEGEIDMLTVMELQDCKYPVVSLGHGASAAKKTCAANYEYFDQFREQIILMFDMDEAGRKAVEEAAQVLPAGKVRVAVLPCKDA

SEQ ID NO: 4 - protein, 115 aa, Mycobacterium tuberculosis
SELYVVEGDSAGGSAKSGRDSMFQAILPLRGKIINVEKARIDRVLKNTEVQAIITALGTGIHDEFDIGKLRYHKIVLMADADVDGQHISTLLLTLLFRFMRPLIENGHVFLAQPP